European Patent Specification EP 3 898 939 B1, published January 25, 2023. Title: Souche Bactérienne Biofertilisante. Applicant: Université de Lorraine INSTITUT NATIONAL DE LA RECHERCHE AGRONOMIQUE. The sequence listing filed with the application follows.

SEQUENCE LISTING (2 sequences)

SEQ ID NO: 1 - DNA, 15 bp, Artificial Sequence
  M13 primer
gagggtggcggttct

SEQ ID NO: 2 - DNA, 10 bp, Artificial Sequence
  RAPD2 primer
agcagcgtgg